European Patent Application EP 4 501 344 A1, published February 5, 2025. Title: Peptide Having Activity of Anti-Inflammation and Anti-Fibrosis and Uses Thereof. Applicant: CAREGEN CO., LTD. Application KR. The sequence listing filed with the application follows.

SEQUENCE LISTING (21 sequences)

SEQ ID NO: 1 - protein, 12 aa, synthetic construct
KYLLVHRPYYRR

SEQ ID NO: 2 - DNA, 21 bp, synthetic construct
  source 1..21: mol_type = other DNA
aacatccaaccttcccaaacg

SEQ ID NO: 3 - DNA, 21 bp, synthetic construct
  source 1..21: mol_type = other DNA
gaccctaagcccccaattctc

SEQ ID NO: 4 - DNA, 20 bp, synthetic construct
  source 1..20: mol_type = other DNA
ttcgacacatgggataacga

SEQ ID NO: 5 - DNA, 20 bp, synthetic construct
  source 1..20: mol_type = other DNA
tctttcaacacgcaggacag

SEQ ID NO: 6 - DNA, 20 bp, synthetic construct
  source 1..20: mol_type = other DNA
aaagaggcactgccagaaaa

SEQ ID NO: 7 - DNA, 20 bp, synthetic construct
  source 1..20: mol_type = other DNA
atctgaggtgcccatgctac

SEQ ID NO: 8 - DNA, 20 bp, synthetic construct
  source 1..20: mol_type = other DNA
gaaggtgcagttttgccaag

SEQ ID NO: 9 - DNA, 20 bp, synthetic construct
  source 1..20: mol_type = other DNA
accctctgcacccagttttc

SEQ ID NO: 10 - DNA, 21 bp, synthetic construct
  source 1..21: mol_type = other DNA
atcattcaccaggcaaattgc

SEQ ID NO: 11 - DNA, 21 bp, synthetic construct
  source 1..21: mol_type = other DNA
ggcttcagcataaagcgtttg

SEQ ID NO: 12 - DNA, 20 bp, synthetic construct
  source 1..20: mol_type = other DNA
gtgatggcatggactgtggt

SEQ ID NO: 13 - DNA, 20 bp, synthetic construct
  source 1..20: mol_type = other DNA
ggagccaaaagggtcatcat

SEQ ID NO: 14 - DNA, 25 bp, synthetic construct
  source 1..25: mol_type = other DNA
ggtgctgtctctctatgcctctgga

SEQ ID NO: 15 - DNA, 25 bp, synthetic construct
  source 1..25: mol_type = other DNA
cccatcaggcaactcgtaactcttc

SEQ ID NO: 16 - DNA, 22 bp, synthetic construct
  source 1..22: mol_type = other DNA
catcacctaccactgcaagaac

SEQ ID NO: 17 - DNA, 18 bp, synthetic construct
  source 1..18: mol_type = other DNA
acgtcgaagccgaattcc

SEQ ID NO: 18 - DNA, 18 bp, synthetic construct
  source 1..18: mol_type = other DNA
ggatgctcctgctgtcac

SEQ ID NO: 19 - DNA, 21 bp, synthetic construct
  source 1..21: mol_type = other DNA
ctgtttgatctggacctgcag

SEQ ID NO: 20 - DNA, 20 bp, synthetic construct
  source 1..20: mol_type = other DNA
ccagcgaccatcaacgcagc

SEQ ID NO: 21 - DNA, 22 bp, synthetic construct
  source 1..22: mol_type = other DNA
ggggcttgttcagtggatgcct